European Patent Application EP 4 442 825 A1, published October 9, 2024. Title: RNA分子. Applicant: 国立大学法人京都大学. The sequence listing filed with the application follows.

SEQUENCE LISTING (57 sequences)

SEQ ID NO: 1 - DNA, 24 bp, synthetic construct
  misc_feature 1..24: note = pIRES2-EGFP_iPCR_Fw
  source 1..24: mol_type = other DNA
tcgagctcaagcttcgaattctgc

SEQ ID NO: 2 - DNA, 22 bp, synthetic construct
  misc_feature 1..22: note = pIRES2-EGFP_iPCR_Rv
  source 1..22: mol_type = other DNA
gctagcggatctgacggttcac

SEQ ID NO: 3 - DNA, 83 bp, synthetic construct
  misc_feature 1..83: note = Rz_N79_code
  source 1..83: mol_type = other DNA
ctgagatgcaggtacatccagctgatgagtcccaaataggacgaaacgcgcttcggtgcgtcctggattccactgctatccac

SEQ ID NO: 4 - DNA, 44 bp, synthetic construct
  misc_feature 1..44: note = InFusion CMV-Rz_N79_Fw
  source 1..44: mol_type = other DNA
gaaccgtcagatccgctagcctgagatgcaggtacatccagctg

SEQ ID NO: 5 - DNA, 74 bp, synthetic construct
  misc_feature 1..74: note = InFusion Rz_N79-AsCas12a_crRNA_Rv
  source 1..74: mol_type = other DNA
aattcgaagcttgagctcgaccggtagatctatctacaagagtagaaattgtggatagcagtggaatccaggac

SEQ ID NO: 6 - DNA, 132 bp, synthetic construct
  misc_feature 1..132: note = InFusion Rz_N79-SaCas9_sgRNA_Rv
  source 1..132: mol_type = other DNA
aattcgaagcttgagctcgaccggtagatctatctcgccaacaagttgacgagataaacacggcattttgccttgttttagtagattctgtttccagagtactaaaacgtggatagcagtggaatccaggac

SEQ ID NO: 7 - DNA, 27 bp, synthetic construct
  misc_feature 1..27: note = XbaI-NLS-SaCas9
  source 1..27: mol_type = other DNA
atatctagagccaccatggccccaaag

SEQ ID NO: 8 - DNA, 36 bp, synthetic construct
  misc_feature 1..36: note = PmeI-3xHA-SaCas9
  source 1..36: mol_type = other DNA
atgtttaaacttaagcgtaatctggaacatcgtatg

SEQ ID NO: 9 - DNA, 28 bp, synthetic construct
  misc_feature 1..28: note = XbaI-AsCpf1
  source 1..28: mol_type = other DNA
atatctagagccaccatgacccagttcg

SEQ ID NO: 10 - DNA, 36 bp, synthetic construct; identical to SEQ ID NO: 8
  misc_feature 1..36: note = PmeI-AsCpf1
  source 1..36: mol_type = other DNA

SEQ ID NO: 11 - DNA, 31 bp, synthetic construct
  misc_feature 1..31: note = TAP_T7_G3C fwd primer
  source 1..31: mol_type = other DNA
cagtgaattgtaatacgactcactatagggc

SEQ ID NO: 12 - DNA, 139 bp, synthetic construct
  misc_feature 1..139: note = 3UTR120A
  source 1..139: mol_type = other DNA
ttttttttttttttttttttttttttttttttttttttttttttttttttttttttttttttttttttttttttttttttttttttttttttttttttttttttttttttttttttttttcctactcaggctttattca

SEQ ID NO: 13 - DNA, 51 bp, synthetic construct
  misc_feature 1..51: note = YF771_T7_5UTR_fwd
  source 1..51: mol_type = other DNA
attgtaatacgactcactatagggcgaattaagagagaaaagaagagtaag

SEQ ID NO: 14 - DNA, 47 bp, synthetic construct
  misc_feature 1..47: note = 5UTR primer for CVB3_IRES
  source 1..47: mol_type = other DNA
gcgaattaagagagaaaagaagagtaagaagaaatataagacaccgg

SEQ ID NO: 15 - DNA, 48 bp, synthetic construct
  misc_feature 1..48: note = Rev3UTR2T20
  source 1..48: mol_type = other DNA
ttttttttttttttttttttcctactcaggctttattcaaagaccaag

SEQ ID NO: 16 - DNA, 76 bp, synthetic construct
  misc_feature 1..76: note = T7-GG-5UTR primer for CVB3_IRES
  source 1..76: mol_type = other DNA
cagtgaattgtaatacgactcactatagggcgaattaagagagaaaagaagagtaagaagaaatataagacaccgg

SEQ ID NO: 17 - DNA, 125 bp, synthetic construct
  misc_feature 1..125: note = T7-G+G+Gluc-Sa_gRNA
  source 1..125: mol_type = other DNA
cagtgaattgtaatacgactcactataggagatcagggcaaacagaacgttttagtactctggaaacagaatctactaaaacaaggcaaaatgccgtgtttatctcgtcaacttgttggcgagat

SEQ ID NO: 18 - DNA, 79 bp, synthetic construct
  misc_feature 1..79: note = Gluc-Sa_gRNA-5UTR primer for CVB3_IRES
  source 1..79: mol_type = other DNA
ccgtgtttatctcgtcaacttgttggcgagatgcgaattaagagagaaaagaagagtaagaagaaatataagacaccgg

SEQ ID NO: 19 - DNA, 119 bp, synthetic construct
  misc_feature 1..119: note = T7-GG+Gluc-AsCas12a_crRNA-5UTR primer for CVB3_IRES
  source 1..119: mol_type = other DNA
cagtgaattgtaatacgactcactataggaatttctactcttgtagatagatcagggcaaacagaactttgagcgaattaagagagaaaagaagagtaagaagaaatataagacaccgg

SEQ ID NO: 20 - DNA, 147 bp, synthetic construct
  misc_feature 1..147: note = T7-GG-5UTR-Gluc-AsCas12a_crRNA for CVB3 IRES
  source 1..147: mol_type = other DNA
cagtgaattgtaatacgactcactatagggcgaattaagagagaaaagaagagtaagaagaaatataagacaccggtcgccaccaatttctactcttgtagatagatcagggcaaacagaactttgattaaaacagcctgtgggttg

SEQ ID NO: 21 - DNA, 102 bp, synthetic construct
  misc_feature 1..102: note = T7-G+Gluc-Sp_gRNA
  source 1..102: mol_type = other DNA
cagtgaattgtaatacgactcactataggagatcagggcaaacagaactgttttagagctagaaatagcaagttaaaataaggctagtccgttatcaacttg

SEQ ID NO: 22 - DNA, 120 bp, synthetic construct
  misc_feature 1..120: note = Gluc-Sp_gRNA-5UTR primer for CVB3_IRES
  source 1..120: mol_type = other DNA
agaaatagcaagttaaaataaggctagtccgttatcaacttgaaaaagtggcaccgagtcggtgcgcgaattaagagagaaaagaagagtaagaagaaatataagacaccggtcgccacc

SEQ ID NO: 23 - DNA, 121 bp, synthetic construct
  misc_feature 1..121: note = T7-G+Gluc-Cj_gRNA
  source 1..121: mol_type = other DNA
cagtgaattgtaatacgactcactataggagatcagggcaaacagaacgttttagtccctgaaaagggactaaaataaagagtttgcgggactctgcggggttacaatcccctaaaaccgc

SEQ ID NO: 24 - DNA, 81 bp, synthetic construct
  misc_feature 1..81: note = Gluc-Cj_gRNA-5UTR primer for CVB3_IRES
  source 1..81: mol_type = other DNA
gcggggttacaatcccctaaaaccgcgcgaattaagagagaaaagaagagtaagaagaaatataagacaccggtcgccacc

SEQ ID NO: 25 - DNA, 144 bp, synthetic construct
  misc_feature 1..144: note = T7-GG+7cx4 Fw
  source 1..144: mol_type = other DNA
ggtctagaaactctcgcctataatcgcgtggatatggcacgcaagtttctaccgggcaccgtaaatgtccgactaggctagaaggtcccaagcccttataaagcagagggaaagatatcacttttaatgctgcctagctccgga

SEQ ID NO: 26 - DNA, 142 bp, synthetic construct
  misc_feature 1..142: note = T7-7cx4 Fw
  source 1..142: mol_type = other DNA
tctagaaactctcgcctataatcgcgtggatatggcacgcaagtttctaccgggcaccgtaaatgtccgactaggctagaaggtcccaagcccttataaagcagagggaaagatatcacttttaatgctgcctagctccgga

SEQ ID NO: 27 - DNA, 144 bp, synthetic construct
  misc_feature 1..144: note = 7cx4_v1 Fw
  source 1..144: mol_type = other DNA
ggtctagaaactctcgcctataatcgcgtggatatggcacgcaagtttctaccgggcaccgtaaatgtccgactaggctagaagtgcccaagcccttataaagcagagggaaagatatcacttttaatgctgcctagctccgga

SEQ ID NO: 28 - DNA, 142 bp, synthetic construct
  misc_feature 1..142: note = 7cx4_v2 Fw
  source 1..142: mol_type = other DNA
ggtagaaactctcgcctataatcgcgtggatatggcacgcaagtttctaccgggcaccgtaaatgtccgactaggctaccagtgcccaagcccttataaagcagagggaaagatatcacttttaatgctgcctagctccgga

SEQ ID NO: 29 - DNA, 110 bp, synthetic construct
  misc_feature 1..110: note = 7cx4_v3 Fw
  source 1..110: mol_type = other DNA
ggtctagaaactctcgcctataatcgcgtggatatggcacgcaagtttctaccgggcaccgtaaatgtccgactaggctagaaggtcccaagcccttgcctagctccgga

SEQ ID NO: 30 - DNA, 108 bp, synthetic construct
  misc_feature 1..108: note = 7cx4_v4 Fw
  source 1..108: mol_type = other DNA
ggtagaaactctcgcctataatcgcgtggatatggcacgcaagtttctaccgggcaccgtaaatgtccgactaggctaccaggtcccaagcccttgcctagctccgga

SEQ ID NO: 31 - DNA, 122 bp, synthetic construct
  misc_feature 1..122: note = T7-G-HCV_1a-CVB3_IRES-EGFP_Fw
  source 1..122: mol_type = other DNA
cagtgaattgtaatacgactcactataggccagccccctgatgggggcgacactccaccatgaatcactcccctggcgaattaagagagaaaagaagagtaagaagaaatataagacaccgg

SEQ ID NO: 32 - DNA, 119 bp, synthetic construct
  misc_feature 1..119: note = T7-GG-HCV_2a-CVB3_IRES-EGFP_Fw
  source 1..119: mol_type = other DNA
cagtgaattgtaatacgactcactataggacctgcccctaataggggcgacactccgccatgaatcactcccgcgaattaagagagaaaagaagagtaagaagaaatataagacaccgg

SEQ ID NO: 33 - DNA, 44 bp, synthetic construct
  misc_feature 1..44: note = AsCas12a ORF_Fw
  source 1..44: mol_type = other DNA
caccggtcgccaccatgacccagttcgagggcttcactaatctg

SEQ ID NO: 34 - DNA, 52 bp, synthetic construct
  misc_feature 1..52: note = AsCas12a ORF_Rv
  source 1..52: mol_type = other DNA
gccccgcagaaggtctagactaagcgtaatctggaacatcgtatgggtaagc

SEQ ID NO: 35 - DNA, 39 bp, synthetic construct
  misc_feature 1..39: note = SaCas9 ORF_Fw
  source 1..39: mol_type = other DNA
caccggtcgccaccatggccccaaagaagaagcggaagg

SEQ ID NO: 36 - DNA, 53 bp, synthetic construct
  misc_feature 1..53: note = SaCas9 ORF_Rv
  source 1..53: mol_type = other DNA
gccccgcagaaggtctagactaagcgtaatctggaacatcgtatgggtaagcg

SEQ ID NO: 37 - DNA, 31 bp, synthetic construct
  misc_feature 1..31: note = CjCas9 ORF_Fw
  source 1..31: mol_type = other DNA
caccggtcgccaccatggccagaatcctggc

SEQ ID NO: 38 - DNA, 44 bp, synthetic construct
  misc_feature 1..44: note = CjCas9 ORF_Rv
  source 1..44: mol_type = other DNA
gccccgcagaaggtctagactaggcgtagtcgggcacgtcgtag

SEQ ID NO: 39 - DNA, 39 bp, synthetic construct
  misc_feature 1..39: note = SphcCas9 ORF fwd primer
  source 1..39: mol_type = other DNA
caccggtcgccaccatggataagaaatacagcattggac

SEQ ID NO: 40 - DNA, 45 bp, synthetic construct
  misc_feature 1..45: note = SphcCas9 ORF rev primer
  source 1..45: mol_type = other DNA
gccccgcagaaggtctagactatcacaccttcctcttcttcttgg

SEQ ID NO: 41 - DNA, 31 bp, synthetic construct; identical to SEQ ID NO: 11
  misc_feature 1..31: note = TAP_T7_G3C fwd primer
  source 1..31: mol_type = other DNA

SEQ ID NO: 42 - DNA, 87 bp, synthetic construct
  misc_feature 1..87: note = IVT_5prime_UTR primer
  source 1..87: mol_type = other DNA
cagtgaattgtaatacgactcactatagggcgaattaagagagaaaagaagagtaagaagaaatataagacaccggtcgccaccatg

SEQ ID NO: 43 - DNA, 37 bp, synthetic construct
  misc_feature 1..37: note = Rev5UTR primer
  source 1..37: mol_type = other DNA
catggtggcgaccggtgtcttatatttcttcttactc

SEQ ID NO: 44 - DNA, 92 bp, synthetic construct
  misc_feature 1..92: note = IVT_3prime_UTR primer
  source 1..92: mol_type = other DNA
tctagaccttctgcggggcttgccttctggccatgcccttcttctctcccttgcacctgtacctcttggtctttgaataaagcctgagtagg

SEQ ID NO: 45 - DNA, 19 bp, synthetic construct
  misc_feature 1..19: note = Fwd3UTR primer
  source 1..19: mol_type = other DNA
tctagaccttctgcggggc

SEQ ID NO: 46 - DNA, 66 bp, synthetic construct
  misc_feature 1..66: note = KWC993_pHHR(6bp)-Sa_gRNA_Rv
  source 1..66: mol_type = other DNA
gacgagcttactcgtttcgtcctcacggactcatcaggttttacgctagcggatctgacggttcac

SEQ ID NO: 47 - DNA, 65 bp, synthetic construct
  misc_feature 1..65: note = KWC994_pHHR(7bp)-Sa_gRNA_Rv
  source 1..65: mol_type = other DNA
gacgagcttactcgtttcgtcctcacggactcatcaggttttagctagcggatctgacggttcac

SEQ ID NO: 48 - DNA, 37 bp, synthetic construct
  misc_feature 1..37: note = KWC995_Sa_gRNA_Fw
  source 1..37: mol_type = other DNA
gttttagtactctggaaacagaatctactaaaacaag

SEQ ID NO: 49 - RNA, 49 nt, synthetic construct
  misc_feature 1..49: note = HHR
  misc_feature 1..6: note = n is a, c, g, or u
  misc_feature 44..49: note = n is a, c, g, or u
  source 1..49: mol_type = other RNA
nnnnnnctgatgagtccgtgaggacgaaacgagtaagctcgtcnnnnnn

SEQ ID NO: 50 - DNA, 160 bp, synthetic construct
  misc_feature 1..160: note = KWC949_Sa_gRNA_anneal
  source 1..160: mol_type = other DNA
cagtgaattgtaatacgactcactataggagatcagggcaaacagaacgttttagtactctggaaacagaatctactaaaacaaggcaaaatgccgtgtttatctcgtcaacttgttggcgagatgcgaattaagagagaaaagaagagtaagaagaaat

SEQ ID NO: 51 - DNA, 160 bp, synthetic construct
  misc_feature 1..160: note = KWC950_Sp_gRNA_anneal
  source 1..160: mol_type = other DNA
cagtgaattgtaatacgactcactataggagatcagggcaaacagaactgttttagagctagaaatagcaagttaaaataaggctagtccgttatcaacttgaaaaagtggcaccgagtcggtgcgcgaattaagagagaaaagaagagtaagaagaaat

SEQ ID NO: 52 - DNA, 55 bp, synthetic construct
  misc_feature 1..55: note = KWC958_Spacer for 3WJdB attachment
  source 1..55: mol_type = other DNA
gcgaattaagagagaaaagaagagtaagaagaaatcccacatactctgatgatcc

SEQ ID NO: 53 - DNA, 160 bp, synthetic construct
  misc_feature 1..160: note = KWC959_Rev primer for 3WJdB attachemnt
  source 1..160: mol_type = other DNA
cccacatacacatggcaagagcccacactctactcgacagatacgaatatctggacccgaccgtctcttgccatgaatgatccgagcccacactctactcgacagatacgaatatctggacccgaccgtctcggatcatcagagtatgtgggatttcttc

SEQ ID NO: 54 - DNA, 160 bp, synthetic construct
  misc_feature 1..160: note = KWC937_Sa_gRNA_temp
  source 1..160: mol_type = other DNA
atttcttcttactcttcttttctctcttaattcgcatctcgccaacaagttgacgagataaacacggcattttgccttgttttagtagattctgtttccagagtactaaaacgttctgtttgccctgatctcctatagtgagtcgtattacaattcactg

SEQ ID NO: 55 - DNA, 160 bp, synthetic construct
  misc_feature 1..160: note = KWC938_Sp_gRNA_temp
  source 1..160: mol_type = other DNA
atttcttcttactcttcttttctctcttaattcgcgcaccgactcggtgccactttttcaagttgataacggactagccttattttaacttgctatttctagctctaaaacagttctgtttgccctgatctcctatagtgagtcgtattacaattcactg

SEQ ID NO: 56 - DNA, 160 bp, synthetic construct; identical to SEQ ID NO: 50
  misc_feature 1..160: note = KWC949_Sa_gRNA_anneal
  source 1..160: mol_type = other DNA

SEQ ID NO: 57 - DNA, 160 bp, synthetic construct; identical to SEQ ID NO: 51
  misc_feature 1..160: note = KWC950_Sp_gRNA_anneal
  source 1..160: mol_type = other DNA